European Patent Application EP 4 245 317 A1, published September 20, 2023. Title: BISPECIFIC ANTIBODY FOR CLAUDIN 18A2 AND CD3 AND APPLICATION OF BISPECIFIC ANTIBODY. Applicant: SHANGHAI QILU PHARMACEUTICAL RESEARCH AND DEVELOPMENT CENTRE LTD. The sequence listing filed with the application follows.

SEQUENCE LISTING (24 sequences)

SEQ ID NO: 1 - protein, 450 aa, Artificial Sequence
  synthetically generated protein
QVQLVQSGAEVKKPGASVKVSCKASGYIFTNYWIHWVRQAPGQGLEWMGRIYPGTGNTYYNEKFTGRVTMTRDTSTSTVYMELSSLRSEDTAVYYCAREGYGKGNSMDYWGQGTTVTVSSASTKGPSVFPLAPSSKSTSGGTAALGCLVKDYFPEPVTVSWNSGALTSGVHTFPAVLQSSGLYSLSSVVTVPSSSLGTQTYICNVNHKPSNTKVDKKVEPKSCDKTHTCPPCPAPEAAGGPSVFLFPPKPKDTLMISRTPEVTCVVVDVSHEDPEVKFNWYVDGVEVHNAKTKPREEQYNSTYRVVSVLTVLHQDWLNGKEYKCKVSNKALPAPIEKTISKAKGQPREPQVYTLPPSRDELTKNQVSLTCLVKGFYPSDIAVEWESNGQPENNYKTTPPVLDSDGSFFLYSKLTVDKSRWQQGNVFSCSVMHEALHNHYTQKSLSLSPGK

SEQ ID NO: 2 - protein, 475 aa, Artificial Sequence
  synthetically generated protein
DIVMTQSPDSLAVSLGERVTMNCKSSQSLLNAGNQKNYLTWYQQKPGQPPKLLFYWASTRESGVPDRFSGSGSGTDFTLTISSVQAEDVAVYHCQNAYYYPYTFGGGTKLEIKRTVAAPSVFIFPPSDEQLKSGTASVVCLLNNFYPREAKVQWKVDNALQSGNSQESVTEQDSKDSTYSLSSTLTLSKADYEKHKVYACEVTHQGLSSPVTKSFNRGECGGGGSAQAVVTQEPSLTVSPGGTVTLTCRSSTGAVTTSNYANWVQQKPGQAPRGLIGGTNKRAPGTPARFSGSLLGGKAALTLSGAQPEDEAEYYCALWYSNLWVFGGGTKLTVLGGGGSGGGGSGGGGSEVKLVESGGGLVQPGGSLKLSCAASGFTFNTYAMNWVRQAPGKGLEWVARIRSKYNNYATYYADSVKDRFTISRDDAKNTLYLQMNNLRTEDTAVYYCVRHGNFGNSYVSWFAYWGQGTLVTVSS

SEQ ID NO: 3 - protein, 715 aa, Artificial Sequence
  synthetically generated protein
QVQLVQSGAEVKKPGASVKVSCKASGYIFTNYWIHWVRQAPGQGLEWMGRIYPGTGNTYYNEKFTGRVTMTRDTSTSTVYMELSSLRSEDTAVYYCAREGYGKGNSMDYWGQGTTVTVSSASTKGPSVFPLAPSSKSTSGGTAALGCLVKDYFPEPVTVSWNSGALTSGVHTFPAVLQSSGLYSLSSVVTVPSSSLGTQTYICNVNHKPSNTKVDKKVEPKSCDKTHTCPPCPAPEAAGGPSVFLFPPKPKDTLMISRTPEVTCVVVDVSHEDPEVKFNWYVDGVEVHNAKTKPREEQYNSTYRVVSVLTVLHQDWLNGKEYKCKVSNKALPAPIEKTISKAKGQPREPQVYTLPPCRDELTKNQVSLWCLVKGFYPSDIAVEWESNGQPENNYKTTPPVLDSDGSFFLYSKLTVDKSRWQQGNVFSCSVMHEALHNHYTQKSLSLSPGAGGGGSGGGGSGGGGSAQAVVTQEPSLTVSPGGTVTLTCRSSTGAVTTSNYANWVQQKPGQAPRGLIGGTNKRAPGTPARFSGSLLGGKAALTLSGAQPEDEAEYYCALWYSNLWVFGGGTKLTVLGGGGSGGGGSGGGGSEVKLVESGGGLVQPGGSLKLSCAASGFTFNTYAMNWVRQAPGKGLEWVARIRSKYNNYATYYADSVKDRFTISRDDAKNTLYLQMNNLRTEDTAVYYCVRHGNFGNSYVSWFAYWGQGTLVTVSS

SEQ ID NO: 4 - protein, 450 aa, Artificial Sequence
  synthetically generated protein
QVQLVQSGAEVKKPGASVKVSCKASGYIFTNYWIHWVRQAPGQGLEWMGRIYPGTGNTYYNEKFTGRVTMTRDTSTSTVYMELSSLRSEDTAVYYCAREGYGKGNSMDYWGQGTTVTVSSASTKGPSVFPLAPSSKSTSGGTAALGCLVKDYFPEPVTVSWNSGALTSGVHTFPAVLQSSGLYSLSSVVTVPSSSLGTQTYICNVNHKPSNTKVDKKVEPKSCDKTHTCPPCPAPEAAGGPSVFLFPPKPKDTLMISRTPEVTCVVVDVSHEDPEVKFNWYVDGVEVHNAKTKPREEQYNSTYRVVSVLTVLHQDWLNGKEYKCKVSNKALPAPIEKTISKAKGQPREPQVCTLPPSRDELTKNQVSLSCAVKGFYPSDIAVEWESNGQPENNYKTTPPVLDSDGSFFLVSKLTVDKSRWQQGNVFSCSVMHEALHNRYTQKSLSLSPGK

SEQ ID NO: 5 - protein, 220 aa, Artificial Sequence
  synthetically generated protein
DIVMTQSPDSLAVSLGERVTMNCKSSQSLLNAGNQKNYLTWYQQKPGQPPKLLFYWASTRESGVPDRFSGSGSGTDFTLTISSVQAEDVAVYHCQNAYYYPYTFGGGTKLEIKRTVAAPSVFIFPPSDEQLKSGTASVVCLLNNFYPREAKVQWKVDNALQSGNSQESVTEQDSKDSTYSLSSTLTLSKADYEKHKVYACEVTHQGLSSPVTKSFNRGEC

SEQ ID NO: 6 - protein, 125 aa, Artificial Sequence
  synthetically generated protein
EVKLVESGGGLVQPGGSLKLSCAASGFTFNTYAMNWVRQAPGKGLEWVARIRSKYNNYATYYADSVKDRFTISRDDAKNTLYLQMNNLRTEDTAVYYCVRHGNFGNSYVSWFAYWGQGTLVTVSS

SEQ ID NO: 7 - protein, 109 aa, Artificial Sequence
  synthetically generated protein
QAVVTQEPSLTVSPGGTVTLTCRSSTGAVTTSNYANWVQQKPGQAPRGLIGGTNKRAPGTPARFSGSLLGGKAALTLSGAQPEDEAEYYCALWYSNLWVFGGGTKLTVL

SEQ ID NO: 8 - protein, 250 aa, Artificial Sequence
  synthetically generated protein
AQAVVTQEPSLTVSPGGTVTLTCRSSTGAVTTSNYANWVQQKPGQAPRGLIGGTNKRAPGTPARFSGSLLGGKAALTLSGAQPEDEAEYYCALWYSNLWVFGGGTKLTVLGGGGSGGGGSGGGGSEVKLVESGGGLVQPGGSLKLSCAASGFTFNTYAMNWVRQAPGKGLEWVARIRSKYNNYATYYADSVKDRFTISRDDAKNTLYLQMNNLRTEDTAVYYCVRHGNFGNSYVSWFAYWGQGTLVTVSS

SEQ ID NO: 9 - protein, 455 aa, Artificial Sequence
  synthetically generated protein
EVKLVESGGGLVQPGGSLKLSCAASGFTFNTYAMNWVRQAPGKGLEWVARIRSKYNNYATYYADSVKDRFTISRDDAKNTLYLQMNNLRTEDTAVYYCVRHGNFGNSYVSWFAYWGQGTLVTVSSASTKGPSVFPLAPSSKSTSGGTAALGCLVKDYFPEPVTVSWNSGALTSGVHTFPAVLQSSGLYSLSSVVTVPSSSLGTQTYICNVNHKPSNTKVDKKVEPKSCDKTHTCPPCPAPEAAGGPSVFLFPPKPKDTLMISRTPEVTCVVVDVSHEDPEVKFNWYVDGVEVHNAKTKPREEQYNSTYRVVSVLTVLHQDWLNGKEYKCKVSNKALPAPIEKTISKAKGQPREPQVYTLPPSRDELTKNQVSLTCLVKGFYPSDIAVEWESNGQPENNYKTTPPVLDSDGSFFLYSKLTVDKSRWQQGNVFSCSVMHEALHNHYTQKSLSLSPGK

SEQ ID NO: 10 - protein, 214 aa, Artificial Sequence
  synthetically generated protein
QAVVTQEPSLTVSPGGTVTLTCRSSTGAVTTSNYANWVQQKPGQAPRGLIGGTNKRAPGTPARFSGSLLGGKAALTLSGAQPEDEAEYYCALWYSNLWVFGGGTKLTVLGQPKANPTVTLFPPSSEELQANKATLVCLISDFYPGAVTVAWKADSSPVKAGVETTTPSKQSNNKYAASSYLSLTPEQWKSHRSYSCQVTHEGSTVEKTVAPTEC

SEQ ID NO: 11 - protein, 5 aa, Artificial Sequence
  synthetically generated protein
NYWIH

SEQ ID NO: 12 - protein, 17 aa, Artificial Sequence
  synthetically generated protein
RIYPGTGNTYYNEKFTG

SEQ ID NO: 13 - protein, 11 aa, Artificial Sequence
  synthetically generated protein
EGYGKGNSMDY

SEQ ID NO: 14 - protein, 17 aa, Artificial Sequence
  synthetically generated protein
KSSQSLLNAGNQKNYLT

SEQ ID NO: 15 - protein, 7 aa, Artificial Sequence
  synthetically generated protein
WASTRES

SEQ ID NO: 16 - protein, 9 aa, Artificial Sequence
  synthetically generated protein
QNAYYYPYT

SEQ ID NO: 17 - protein, 5 aa, Artificial Sequence
  synthetically generated protein
TYAMN

SEQ ID NO: 18 - protein, 19 aa, Artificial Sequence
  synthetically generated protein
RIRSKYNNYATYYADSVKD

SEQ ID NO: 19 - protein, 14 aa, Artificial Sequence
  synthetically generated protein
HGNFGNSYVSWFAY

SEQ ID NO: 20 - protein, 14 aa, Artificial Sequence
  synthetically generated protein
RSSTGAVTTSNYAN

SEQ ID NO: 21 - protein, 7 aa, Artificial Sequence
  synthetically generated protein
GTNKRAP

SEQ ID NO: 22 - protein, 9 aa, Artificial Sequence
  synthetically generated protein
ALWYSNLWV

SEQ ID NO: 23 - protein, 120 aa, Artificial Sequence
  synthetically generated protein
QVQLVQSGAEVKKPGASVKVSCKASGYIFTNYWIHWVRQAPGQGLEWMGRIYPGTGNTYYNEKFTGRVTMTRDTSTSTVYMELSSLRSEDTAVYYCAREGYGKGNSMDYWGQGTTVTVSS

SEQ ID NO: 24 - protein, 113 aa, Artificial Sequence
  synthetically generated protein
DIVMTQSPDSLAVSLGERVTMNCKSSQSLLNAGNQKNYLTWYQQKPGQPPKLLFYWASTRESGVPDRFSGSGSGTDFTLTISSVQAEDVAVYHCQNAYYYPYTFGGGTKLEIK